European Patent Specification EP 3 464 322 B1, published April 5, 2023. Title: NOVEL MOLECULES FOR THE TREATMENT OF INFLAMMATION. Applicant: Tel HaShomer Medical Research Infrastructure and Services Ltd. MAGGIO, Nicola CHAPMAN, Joab SHAVIT STEIN, Efrat. The sequence listing filed with the application follows.

SEQUENCE LISTING (59 sequences)

SEQ ID NO: 1 - protein, 4 aa, Artificial sequence
  Synthetic peptide
  MISC_FEATURE (1)..(1): N-terminal modification: Tosyl  or other peptidase activity protecting moiety
  MISC_FEATURE (4)..(4): C-terminal modification: Amide or other stabilizing moiety
ANSF

SEQ ID NO: 2 - protein, 4 aa, Artificial sequence
  Synthetic peptide
  MISC_FEATURE (1)..(1): N-terminal modification: Tosyl  or other peptidase activity protecting moiety
  MISC_FEATURE (4)..(4): C-terminal modification: Amide or other stabilizing moiety
ANAF

SEQ ID NO: 3 - protein, 9 aa, Artificial sequence
  Synthetic peptide
  MISC_FEATURE (1)..(1): N-terminal modification: Tosyl  or other peptidase activity protecting moiety
  MISC_FEATURE (6)..(7): may be gamma-carboxylated
  MISC_FEATURE (9)..(9): C-terminal modification: Amide or other stabilizing moiety
ANSFLEELR

SEQ ID NO: 4 - protein, 9 aa, Artificial sequence
  Synthetic peptide
  MISC_FEATURE (1)..(1): N-terminal modification: Tosyl  or other peptidase activity protecting moiety
  MISC_FEATURE (6)..(7): may be gamma-carboxylated
  MISC_FEATURE (9)..(9): C-terminal modification: Amide or other stabilizing moiety
ANAFLEELR

SEQ ID NO: 5 - protein, 4 aa, Artificial sequence
  Synthetic peptide
  MISC_FEATURE (1)..(1): N-terminal modification: Tosyl  or other peptidase activity protecting moiety
  MISC_FEATURE (1)..(2): may be gamma-carboxylated
  MISC_FEATURE (4)..(4): C-terminal modification: Amide or other stabilizing moiety
EEAK

SEQ ID NO: 6 - protein, 4 aa, Artificial sequence
  Synthetic peptide
  MISC_FEATURE (1)..(1): N-terminal modification: Tosyl  or other peptidase activity protecting moiety
  MISC_FEATURE (1)..(2): may be gamma-carboxylated
  MISC_FEATURE (4)..(4): C-terminal modification: Amide or other stabilizing moiety
EEAR

SEQ ID NO: 7 - protein, 7 aa, Artificial sequence
  Synthetic peptide
  MISC_FEATURE (1)..(1): N-terminal modification: Tosyl  or other peptidase activity protecting moiety
  MISC_FEATURE (1)..(2): may be gamma-carboxylated
  MISC_FEATURE (5)..(5): may be gamma-carboxylated
  MISC_FEATURE (7)..(7): C-terminal modification: Amide or other stabilizing moiety
EEAKEIF

SEQ ID NO: 8 - protein, 7 aa, Artificial sequence
  Synthetic peptide
  MISC_FEATURE (1)..(1): N-terminal modification: Tosyl  or other peptidase activity protecting moiety
  MISC_FEATURE (1)..(2): may be gamma-carboxylated
  MISC_FEATURE (5)..(5): may be gamma-carboxylated
  MISC_FEATURE (7)..(7): C-terminal modification: Amide or other stabilizing moiety
EEAREIF

SEQ ID NO: 9 - DNA, 20 bp, Artificial sequence
  Single strand DNA oligonucleotide
ccgaaagggcaacctagagc

SEQ ID NO: 10 - DNA, 19 bp, Artificial sequence
  Single strand DNA oligonucleotide
ggcccagaacacgtctgtg

SEQ ID NO: 11 - DNA, 16 bp, Artificial sequence
  Single strand DNA oligonucleotide
gtggccgggaatgcaa

SEQ ID NO: 12 - DNA, 25 bp, Artificial sequence
  Single strand DNA oligonucleotide
aacccttcattgtcttcgttaatga

SEQ ID NO: 13 - DNA, 22 bp, Artificial sequence
  Single strand DNA oligonucleotide
accgtgaggcttggtgagtatg

SEQ ID NO: 14 - DNA, 20 bp, Artificial sequence
  Single strand DNA oligonucleotide
acgcactcatttcgagcaac

SEQ ID NO: 15 - DNA, 21 bp, Artificial sequence
  Single strand DNA oligonucleotide
tgaacccccgctcattctttc

SEQ ID NO: 16 - DNA, 22 bp, Artificial sequence
  Single strand DNA oligonucleotide
ccagcaggacgctttcattttt

SEQ ID NO: 17 - DNA, 23 bp, Artificial sequence
  Single strand DNA oligonucleotide
tgaaagacttgctcgagatgtca

SEQ ID NO: 18 - DNA, 20 bp, Artificial sequence
  Single strand DNA oligonucleotide
cacacagagggccacaatgt

SEQ ID NO: 19 - protein, 9 aa, Artificial sequence
  Isolated peptide
  MISC_FEATURE (1)..(1): N-terminal modification: Tosyl  or other peptidase activity protecting moiety
  MISC_FEATURE (6)..(7): may be gamma-carboxylated
  MISC_FEATURE (9)..(9): C-terminal modification: Amide or other stabilizing moiety
ANSFLEEMK

SEQ ID NO: 20 - protein, 7 aa, Artificial sequence
  Isolated peptide
  MISC_FEATURE (1)..(1): N-terminal modification: Tosyl  or other peptidase activity protecting moiety
  MISC_FEATURE (1)..(2): may be gamma-carboxylated
  MISC_FEATURE (5)..(5): may be gamma-carboxylated
  MISC_FEATURE (7)..(7): C-terminal modification: Amide or other stabilizing moiety
EEAREVF

SEQ ID NO: 21 - protein, 9 aa, Artificial sequence
  Isolated peptide
  MISC_FEATURE (1)..(1): N-terminal modification: Tosyl  or other peptidase activity protecting moiety
  MISC_FEATURE (6)..(7): may be gamma-carboxylated
  MISC_FEATURE (9)..(9): C-terminal modification: Amide or other stabilizing moiety
ANTFLEEVR

SEQ ID NO: 22 - protein, 7 aa, Artificial sequence
  Isolated peptide
  MISC_FEATURE (1)..(1): N-terminal modification: Tosyl  or other peptidase activity protecting moiety
  MISC_FEATURE (1)..(2): may be gamma-carboxylated
  MISC_FEATURE (5)..(5): may be gamma-carboxylated
  MISC_FEATURE (7)..(7): C-terminal modification: Amide or other stabilizing moiety
EEAFEAL

SEQ ID NO: 23 - protein, 9 aa, Artificial sequence
  Isolated peptide
  MISC_FEATURE (1)..(1): N-terminal modification: Tosyl  or other peptidase activity protecting moiety
  MISC_FEATURE (6)..(7): may be gamma-carboxylated
  MISC_FEATURE (9)..(9): C-terminal modification: Amide or other stabilizing moiety
NSGKLEEFV

SEQ ID NO: 24 - protein, 7 aa, Artificial sequence
  Isolated peptide
  MISC_FEATURE (1)..(1): N-terminal modification: Tosyl  or other peptidase activity protecting moiety
  MISC_FEATURE (1)..(2): may be gamma-carboxylated
  MISC_FEATURE (5)..(5): may be gamma-carboxylated
  MISC_FEATURE (7)..(7): C-terminal modification: Amide or other stabilizing moiety
EEAREVF

SEQ ID NO: 25 - protein, 9 aa, Artificial sequence
  Isolated peptide
  MISC_FEATURE (1)..(1): N-terminal modification: Tosyl  or other peptidase activity protecting moiety
  MISC_FEATURE (6)..(7): may be gamma-carboxylated
  MISC_FEATURE (9)..(9): C-terminal modification: Amide or other stabilizing moiety
ANSLLEETK

SEQ ID NO: 26 - protein, 7 aa, Artificial sequence
  Isolated peptide
  MISC_FEATURE (1)..(1): N-terminal modification: Tosyl  or other peptidase activity protecting moiety
  MISC_FEATURE (1)..(2): may be gamma-carboxylated
  MISC_FEATURE (5)..(5): may be gamma-carboxylated
  MISC_FEATURE (7)..(7): C-terminal modification: Amide or other stabilizing moiety
EEAREVF

SEQ ID NO: 27 - protein, 9 aa, Artificial sequence
  Isolated peptide
  MISC_FEATURE (1)..(1): N-terminal modification: Tosyl  or other peptidase activity protecting moiety
  MISC_FEATURE (6)..(7): may be gamma-carboxylated
  MISC_FEATURE (9)..(9): C-terminal modification: Amide or other stabilizing moiety
GSYLLEELF

SEQ ID NO: 28 - protein, 7 aa, Artificial sequence
  Isolated peptide
  MISC_FEATURE (1)..(1): N-terminal modification: Tosyl  or other peptidase activity protecting moiety
  MISC_FEATURE (1)..(2): may be gamma-carboxylated
  MISC_FEATURE (5)..(5): may be gamma-carboxylated
  MISC_FEATURE (7)..(7): C-terminal modification: Amide or other stabilizing moiety
EEAREVF

SEQ ID NO: 29 - protein, 4 aa, Artificial sequence
  Isolated peptide
  MISC_FEATURE (1)..(1): N-terminal modification: Tosyl  or other peptidase activity protecting moiety
  MISC_FEATURE (4)..(4): C-terminal modification: Amide or other stabilizing moiety
ANTF

SEQ ID NO: 30 - protein, 4 aa, Artificial sequence
  Isolated peptide
  MISC_FEATURE (1)..(1): N-terminal modification: Tosyl  or other peptidase activity protecting moiety
  MISC_FEATURE (1)..(2): may be gamma-carboxylated
  MISC_FEATURE (4)..(4): C-terminal modification: Amide or other stabilizing moiety
EEAF

SEQ ID NO: 31 - protein, 4 aa, Artificial sequence
  Isolated peptide
  MISC_FEATURE (1)..(1): N-terminal modification: Tosyl  or other peptidase activity protecting moiety
  MISC_FEATURE (4)..(4): C-terminal modification: Amide or other stabilizing moiety
NSGK

SEQ ID NO: 32 - protein, 4 aa, Artificial sequence
  Isolated peptide
  MISC_FEATURE (1)..(1): N-terminal modification: Tosyl  or other peptidase activity protecting moiety
  MISC_FEATURE (4)..(4): C-terminal modification: Amide or other stabilizing moiety
ANSL

SEQ ID NO: 33 - protein, 4 aa, Artificial sequence
  Isolated peptide
  MISC_FEATURE (1)..(1): N-terminal modification: Tosyl  or other peptidase activity protecting moiety
  MISC_FEATURE (4)..(4): C-terminal modification: Amide or other stabilizing moiety
GSYL

SEQ ID NO: 34 - protein, 3 aa, Artificial sequence
  Isolated peptide
  MISC_FEATURE (1)..(1): N-terminal modification: Tosyl  or other peptidase activity protecting moiety
  MISC_FEATURE (3)..(3): C-terminal modification: Amide or other stabilizing moiety
ANS

SEQ ID NO: 35 - protein, 3 aa, Artificial sequence
  Isolated peptide
  MISC_FEATURE (1)..(1): N-terminal modification: Tosyl  or other peptidase activity protecting moiety
  MISC_FEATURE (3)..(3): C-terminal modification: Amide or other stabilizing moiety
NSF

SEQ ID NO: 36 - protein, 3 aa, Artificial sequence
  Isolated peptide
  MISC_FEATURE (1)..(1): N-terminal modification: Tosyl  or other peptidase activity protecting moiety
  MISC_FEATURE (3)..(3): C-terminal modification: Amide or other stabilizing moiety
SFL

SEQ ID NO: 37 - protein, 3 aa, Artificial sequence
  Isolated peptide
  MISC_FEATURE (1)..(1): N-terminal modification: Tosyl  or other peptidase activity protecting moiety
  MISC_FEATURE (3)..(3): C-terminal modification: Amide or other stabilizing moiety
  MISC_FEATURE (3)..(3): may be gamma-carboxylated
FLE

SEQ ID NO: 38 - protein, 3 aa, Artificial sequence
  Isolated peptide
  MISC_FEATURE (1)..(1): N-terminal modification: Tosyl  or other peptidase activity protecting moiety
  MISC_FEATURE (2)..(3): may be gamma-carboxylated
  MISC_FEATURE (3)..(3): C-terminal modification: Amide or other stabilizing moiety
LEE

SEQ ID NO: 39 - protein, 3 aa, Artificial sequence
  Isolated peptide
  MISC_FEATURE (1)..(1): N-terminal modification: Tosyl  or other peptidase activity protecting moiety
  MISC_FEATURE (1)..(2): may be gamma-carboxylated
  MISC_FEATURE (3)..(3): C-terminal modification: Amide or other stabilizing moiety
EEL

SEQ ID NO: 40 - protein, 3 aa, Artificial sequence
  Isolated peptide
  MISC_FEATURE (1)..(1): N-terminal modification: Tosyl  or other peptidase activity protecting moiety
  MISC_FEATURE (1)..(1): may be gamma-carboxylated
  MISC_FEATURE (3)..(3): C-terminal modification: Amide or other stabilizing moiety
ELR

SEQ ID NO: 41 - protein, 3 aa, Artificial sequence
  Isolated peptide
  MISC_FEATURE (1)..(1): N-terminal modification: Tosyl  or other peptidase activity protecting moiety
  MISC_FEATURE (3)..(3): C-terminal modification: Amide or other stabilizing moiety
ANA

SEQ ID NO: 42 - protein, 3 aa, Artificial sequence
  Isolated peptide
  MISC_FEATURE (1)..(1): N-terminal modification: Tosyl  or other peptidase activity protecting moiety
  MISC_FEATURE (3)..(3): C-terminal modification: Amide or other stabilizing moiety
NAF

SEQ ID NO: 43 - protein, 3 aa, Artificial sequence
  Isolated peptide
  MISC_FEATURE (1)..(1): N-terminal modification: Tosyl  or other peptidase activity protecting moiety
  MISC_FEATURE (3)..(3): C-terminal modification: Amide or other stabilizing moiety
AFL

SEQ ID NO: 44 - protein, 3 aa, Artificial sequence
  Isolated peptide
  MISC_FEATURE (1)..(1): N-terminal modification: Tosyl  or other peptidase activity protecting moiety
  MISC_FEATURE (1)..(2): may be gamma-carboxylated
  MISC_FEATURE (3)..(3): C-terminal modification: Amide or other stabilizing moiety
EEA

SEQ ID NO: 45 - protein, 3 aa, Artificial sequence
  Isolated peptide
  MISC_FEATURE (1)..(1): N-terminal modification: Tosyl  or other peptidase activity protecting moiety
  MISC_FEATURE (1)..(1): may be gamma-carboxylated
  MISC_FEATURE (3)..(3): C-terminal modification: Amide or other stabilizing moiety
EAK

SEQ ID NO: 46 - protein, 3 aa, Artificial sequence
  Isolated peptide
  MISC_FEATURE (1)..(1): N-terminal modification: Tosyl  or other peptidase activity protecting moiety
  MISC_FEATURE (3)..(3): C-terminal modification: Amide or other stabilizing moiety
  MISC_FEATURE (3)..(3): may be gamma-carboxylated
AKE

SEQ ID NO: 47 - protein, 3 aa, Artificial sequence
  Isolated peptide
  MISC_FEATURE (1)..(1): N-terminal modification: Tosyl  or other peptidase activity protecting moiety
  MISC_FEATURE (2)..(2): may be gamma-carboxylated
  MISC_FEATURE (3)..(3): C-terminal modification: Amide or other stabilizing moiety
KEI

SEQ ID NO: 48 - protein, 3 aa, Artificial sequence
  Isolated peptide
  MISC_FEATURE (1)..(1): N-terminal modification: Tosyl  or other peptidase activity protecting moiety
  MISC_FEATURE (1)..(1): may be gamma-carboxylated
  MISC_FEATURE (3)..(3): C-terminal modification: Amide or other stabilizing moiety
EIF

SEQ ID NO: 49 - protein, 3 aa, Artificial sequence
  Isolated peptide
  MISC_FEATURE (1)..(1): N-terminal modification: Tosyl  or other peptidase activity protecting moiety
  MISC_FEATURE (1)..(1): may be gamma-carboxylated
  MISC_FEATURE (3)..(3): C-terminal modification: Amide or other stabilizing moiety
EAR

SEQ ID NO: 50 - protein, 3 aa, Artificial sequence
  Isolated peptide
  MISC_FEATURE (1)..(1): N-terminal modification: Tosyl  or other peptidase activity protecting moiety
  MISC_FEATURE (3)..(3): C-terminal modification: Amide or other stabilizing moiety
  MISC_FEATURE (3)..(3): may be gamma-carboxylated
ARE

SEQ ID NO: 51 - protein, 3 aa, Artificial Sequence
  Isolated peptide
  MISC_FEATURE (1)..(1): N-terminal modification: Tosyl  or other peptidase activity protecting moiety
  MISC_FEATURE (2)..(2): may be gamma-carboxylated
  MISC_FEATURE (3)..(3): C-terminal modification: Amide or other stabilizing moiety
REI

SEQ ID NO: 52 - protein, 4 aa, Artificial Sequence
  Isolated peptide
  MISC_FEATURE (1)..(1): N-terminal modification: Tosyl  or other peptidase activity protecting moiety
  MISC_FEATURE (1)..(1): X can be either Gly, Ala, Val, Leu or Ile
  MISC_FEATURE (2)..(2): X can be either Asp, Glu, Lys, Arg, His, Asn, Gln, Ser, Thr, Tyr or Cys
  MISC_FEATURE (2)..(3): may be gamma-carboxylated
  MISC_FEATURE (2)..(2): may be gamma-carboxylated
  misc_feature (3)..(3): Xaa can be any naturally occurring amino acid
  MISC_FEATURE (4)..(4): C-terminal modification: Amide or other stabilizing moiety
  MISC_FEATURE (4)..(4): X can be either Gly, Ala, Val, Leu, Ile, Phe, Trp, Pro, Met, Phe, Tyr or Trp
XXXX

SEQ ID NO: 53 - protein, 4 aa, Artificial Sequence
  Isolated peptide
  MISC_FEATURE (1)..(1): N-terminal modification: Tosyl  or other peptidase activity protecting moiety
  MISC_FEATURE (1)..(2): X is an acidic polar amino acid: Asp or  Glu
  MISC_FEATURE (1)..(2): may be gamma-carboxylated
  MISC_FEATURE (3)..(3): X  is a non-polar, aliphatic amino acid: Gly, Ala, Val, Leu or Ile
  MISC_FEATURE (4)..(4): C-terminal modification: Amide or other stabilizing moiety
  MISC_FEATURE (4)..(4): may be gamma-carboxylated
  misc_feature (4)..(4): Xaa can be any naturally occurring amino acid
XXXX

SEQ ID NO: 54 - DNA, 20 bp, Artificial sequence
  Single strand DNA oligonucleotide
cctatgagccagccagaatc

SEQ ID NO: 55 - DNA, 20 bp, Artificial sequence
  Single strand DNA oligonucleotide
gcaggacgctttcatttttc

SEQ ID NO: 56 - DNA, 20 bp, Artificial sequence
  Single strand DNA oligonucleotide
gcagctcaatgcctacaacc

SEQ ID NO: 57 - DNA, 21 bp, Artificial sequence
  Single strand DNA oligonucleotide
ctgtttggctccctttcatgt

SEQ ID NO: 58 - DNA, 21 bp, Artificial sequence
  Single strand DNA oligonucleotide
agatggatagtgaccgcaagc

SEQ ID NO: 59 - DNA, 21 bp, Artificial sequence
  Single strand DNA oligonucleotide
gtcatgttcacccatcaccac